European Patent Specification EP 3 591 049 B1, published November 22, 2023. Title: Horseshoe crab factor B variant. Applicant: Seikagaku Corporation. The sequence listing filed with the application follows.

SEQUENCE LISTING (42 sequences)

SEQ ID NO: 1 - DNA, 1203 bp, Tachypleus tridentatus
  Tachypleus tridentatus factor B
atgacgtggatatgtgtgataacgttgtttgctctggcttctgctacgttgggtaacaaagttagtagagtgggggtcctcttccccaagacacggaacgacaatgagtgtacagcaagagggggattgaaaggatcctgcaaatccctcatagactgtcctagtgtcttggctacgttgaaggacagttttcctgtcgtttgctcttggaatggtcgatttcagcctattgtctgctgtcctgatgcaatagcaccaccacctgtaaccacaacagctgtaactgtaatatctacaaaagaaccaaagcttccaagattacatatatcaggttgtggaaaaagaaaagtcaaaatagatattacaactgttggacgctctggatcaccaatacttcctccgatatctactcctcaaaattcaacaggtgggagaggaattattgctggaggcgtagaagccaaaattggcgcgtggccttggatggcagctgtttttgtgaaaaactttggcattggcagattccactgtgctggtagcataatcagtaacaagtacattttgtcagctgcccacgccttccttatcggaggtcgaaagttgaccccaactcgcttagctgtccgtgtgggaggccactacataaagaggggtcaagagtatccagtgaaagacgtgattatccatcctcattatgtagaaaaggagaactacaatgatatagccataatcgagttaaaagaggaactgaactttacggacttggtcaatcctatatgtctccctgatccagagacagtaacggatccattaaaagacagaattgtgactgcagcgggatggggcgatctggatttctccggtccacggagccaagttctacgtgaggtaagcatcccagttgttccagttgataaatgtgatcaagcctatgagaaactcaacaccccttcactaaaaaatgggataacgaataacttcctttgcgctggattggaagaaggagggaaagacgcttgccaaggcgattctggtggaccgttgatgctagtgaacaacactaggtggatagtagtaggagttgtgtcgttcgggcacaagtgtgccgaggaaggatatcctggtgtgtactcgcgcgtagcgagttacctagactggatcgcgaaagttacgaactcgttagatcatgccgtcactaactga

SEQ ID NO: 2 - protein, 400 aa, Tachypleus tridentatus
  Tachypleus tridentatus factor B
MTWICVITLFALASATLGNKVSRVGVLFPKTRNDNECTARGGLKGSCKSLIDCPSVLATLKDSFPVVCSWNGRFQPIVCCPDAIAPPPVTTTAVTVISTKEPKLPRLHISGCGKRKVKIDITTVGRSGSPILPPISTPQNSTGGRGIIAGGVEAKIGAWPWMAAVFVKNFGIGRFHCAGSIISNKYILSAAHAFLIGGRKLTPTRLAVRVGGHYIKRGQEYPVKDVIIHPHYVEKENYNDIAIIELKEELNFTDLVNPICLPDPETVTDPLKDRIVTAAGWGDLDFSGPRSQVLREVSIPVVPVDKCDQAYEKLNTPSLKNGITNNFLCAGLEEGGKDACQGDSGGPLMLVNNTRWIVVGVVSFGHKCAEEGYPGVYSRVASYLDWIAKVTNSLDHAVTN

SEQ ID NO: 3 - DNA, 1203 bp, Limulus polyphemus
  Limulus polyphemus factor B
atggcgtggatttgtgtgataacgttgtttgctttggcttctagtacgttgagtaataaagttagtagagtggggatcatctttcctaagacacagaacgataataaacagtgtacagcaaaaggtggattaaaagggtcctgcaagtccctcacagactgtcctgctgtcttggctacgttgaaggatagtttccctgtcgtttgctcttggaatggtcggtttcagcctattgtatgttgtcctgatgcagcagcaccaagtgtaaccacaacagttacaactattgtccctacaaaagaaacaaagattccaagattacatataccaggttgtggaaaaagaaaagtaaatgtagatattacaactattggacgttcggggtcaccaatacttcctcccatatctacttctcaagatttgaagggtgggagaggaatcattgctggaggtgtagaagctaaaattggcgcctggccttggatggcagctgtttttgtgaaaaattttggcattggcagattccattgtgctggtagcataatcagtagcaagtacattttgtctgctgcccacgctttcctcattggaggtcgaaagctgaccccaactcgcttagctgtccgcgtaggaggccactacgtaaagatgggtcaagaatatcatgtggaagatgtgattatccatcctgactacgtagaaagggagaattacaatgatattgctatcattgtgttaaaagaggaactgaattttactgatttggtccgtccaatctgtctccctgacccagaggcagtaacagattcattaaaaggcagaagggtgacagtagctggatggggtgatctggatttcgccggtccacgaagtcaagttctgcgcgaggttagtatccccgttgttccaatcggtgactgtaacaaagcctatcagaagctcaacacccttgctcttaaaaatgggataacgaaaaagtttatttgtgctggattggaagaaggtgggaaagatgcttgtcaaggcgattctggtggaccgttgatgctagtgaacaatagtagttggatagtgacgggagtggtgtcgttcggacacaagtgtgccgaagagggatttcctggtgtgtacacgcgtgtagtgagttacctagagtggatcgcgaaggttacgaactcgttagaccagacagtcactaactga

SEQ ID NO: 4 - protein, 400 aa, Limulus polyphemus
  Limulus polyphemus factor B
MAWICVITLFALASSTLSNKVSRVGIIFPKTQNDNKQCTAKGGLKGSCKSLTDCPAVLATLKDSFPVVCSWNGRFQPIVCCPDAAAPSVTTTVTTIVPTKETKIPRLHIPGCGKRKVNVDITTIGRSGSPILPPISTSQDLKGGRGIIAGGVEAKIGAWPWMAAVFVKNFGIGRFHCAGSIISSKYILSAAHAFLIGGRKLTPTRLAVRVGGHYVKMGQEYHVEDVIIHPDYVERENYNDIAIIVLKEELNFTDLVRPICLPDPEAVTDSLKGRRVTVAGWGDLDFAGPRSQVLREVSIPVVPIGDCNKAYQKLNTLALKNGITKKFICAGLEEGGKDACQGDSGGPLMLVNNSSWIVTGVVSFGHKCAEEGFPGVYTRVVSYLEWIAKVTNSLDQTVTN

SEQ ID NO: 5 - DNA, 1203 bp, Artificial Sequence
  Tachypleus tridentatus factor B variant
atgacgtggatatgtgtgataacgttgtttgctctggcttctgctacgttgggtaacaaagttagtagagtgggggtcctcttccccaagacacggaacgacaatgagtgtacagcaagagggggattgaaaggatcctgcaaatccctcatagactgtcctagtgtcttggctacgttgaaggacagttttcctgtcgtttgctcttggaatggtcgatttcagcctattgtctgctgtcctgatgcaatagcaccaccacctgtaaccacaacagctgtaactgtaatatctacaaaagaaccaaagcttccaagattacatatatcaggttgtggaaaaagaaaagtcaaaatagatattacaactgttggacgctctggatcaccaatacttcctccgatatctactcctcaaaattcaacaggtgggagaggaattattgctggaggcgtagaagccaaaattggcgcgtggccttggatggcagctgtttttgtgaaaaactttggcattggcagattccactgtgctggtagcataatcagtaacaagtacattttgtcagctgcccactgtttccttatcggaggtcgaaagttgaccccaactcgcttagctgtccgtgtgggaggccactacataaagaggggtcaagagtatccagtgaaagacgtgattatccatcctcattatgtagaaaaggagaactacaatgatatagccataatcgagttaaaagaggaactgaactttacggacttggtcaatcctatatgtctccctgatccagagacagtaacggatccattaaaagacagaattgtgactgcagcgggatggggcgatctggatttctccggtccacggagccaagttctacgtgaggtaagcatcccagttgttccagttgataaatgtgatcaagcctatgagaaactcaacaccccttcactaaaaaatgggataacgaataacttcctttgcgctggattggaagaaggagggaaagacgcttgccaaggcgattctggtggaccgttgatgctagtgaacaacactaggtggatagtagtaggagttgtgtcgttcgggcacaagtgtgccgaggaaggatatcctggtgtgtactcgcgcgtagcgagttacctagactggatcgcgaaagttacgaactcgttagatcatgccgtcactaactga

SEQ ID NO: 6 - DNA, 1203 bp, Artificial Sequence
  Tachypleus tridentatus factor B variant
atgacgtggatatgtgtgataacgttgtttgctctggcttctgctacgttgggtaacaaagttagtagagtgggggtcctcttccccaagacacggaacgacaatgagtgtacagcaagagggggattgaaaggatcctgcaaatccctcatagactgtcctagtgtcttggctacgttgaaggacagttttcctgtcgtttgctcttggaatggtcgatttcagcctattgtctgctgtcctgatgcaatagcaccaccacctgtaaccacaacagctgtaactgtaatatctacaaaagaaccaaagcttccaagattacatatatcaggttgtggaaaaagaaaagtcaaaatagatattacaactgttggacgctctggatcaccaatacttcctccgatatctactcctcaaaattcaacaggtgggagaggaattattgctggaggcgtagaagccaaaattggcgcgtggccttggatggcagctgtttttgtgaaaaactttggcattggcagattccactgtgctggtagcataatcagtaacaagtacattttgtcagctgcccactgcttccttatcggaggtcgaaagttgaccccaactcgcttagctgtccgtgtgggaggccactacataaagaggggtcaagagtatccagtgaaagacgtgattatccatcctcattatgtagaaaaggagaactacaatgatatagccataatcgagttaaaagaggaactgaactttacggacttggtcaatcctatatgtctccctgatccagagacagtaacggatccattaaaagacagaattgtgactgcagcgggatggggcgatctggatttctccggtccacggagccaagttctacgtgaggtaagcatcccagttgttccagttgataaatgtgatcaagcctatgagaaactcaacaccccttcactaaaaaatgggataacgaataacttcctttgcgctggattggaagaaggagggaaagacgcttgccaaggcgattctggtggaccgttgatgctagtgaacaacactaggtggatagtagtaggagttgtgtcgttcgggcacaagtgtgccgaggaaggatatcctggtgtgtactcgcgcgtagcgagttacctagactggatcgcgaaagttacgaactcgttagatcatgccgtcactaactga

SEQ ID NO: 7 - protein, 400 aa, Artificial Sequence
  Tachypleus tridentatus factor B variant
MTWICVITLFALASATLGNKVSRVGVLFPKTRNDNECTARGGLKGSCKSLIDCPSVLATLKDSFPVVCSWNGRFQPIVCCPDAIAPPPVTTTAVTVISTKEPKLPRLHISGCGKRKVKIDITTVGRSGSPILPPISTPQNSTGGRGIIAGGVEAKIGAWPWMAAVFVKNFGIGRFHCAGSIISNKYILSAAHCFLIGGRKLTPTRLAVRVGGHYIKRGQEYPVKDVIIHPHYVEKENYNDIAIIELKEELNFTDLVNPICLPDPETVTDPLKDRIVTAAGWGDLDFSGPRSQVLREVSIPVVPVDKCDQAYEKLNTPSLKNGITNNFLCAGLEEGGKDACQGDSGGPLMLVNNTRWIVVGVVSFGHKCAEEGYPGVYSRVASYLDWIAKVTNSLDHAVTN

SEQ ID NO: 8 - DNA, 1203 bp, Artificial Sequence
  Limulus polyphemus factor B variant
atggcgtggatttgtgtgataacgttgtttgctttggcttctagtacgttgagtaataaagttagtagagtggggatcatctttcctaagacacagaacgataataaacagtgtacagcaaaaggtggattaaaagggtcctgcaagtccctcacagactgtcctgctgtcttggctacgttgaaggatagtttccctgtcgtttgctcttggaatggtcggtttcagcctattgtatgttgtcctgatgcagcagcaccaagtgtaaccacaacagttacaactattgtccctacaaaagaaacaaagattccaagattacatataccaggttgtggaaaaagaaaagtaaatgtagatattacaactattggacgttcggggtcaccaatacttcctcccatatctacttctcaagatttgaagggtgggagaggaatcattgctggaggtgtagaagctaaaattggcgcctggccttggatggcagctgtttttgtgaaaaattttggcattggcagattccattgtgctggtagcataatcagtagcaagtacattttgtctgctgcccactgtttcctcattggaggtcgaaagctgaccccaactcgcttagctgtccgcgtaggaggccactacgtaaagatgggtcaagaatatcatgtggaagatgtgattatccatcctgactacgtagaaagggagaattacaatgatattgctatcattgtgttaaaagaggaactgaattttactgatttggtccgtccaatctgtctccctgacccagaggcagtaacagattcattaaaaggcagaagggtgacagtagctggatggggtgatctggatttcgccggtccacgaagtcaagttctgcgcgaggttagtatccccgttgttccaatcggtgactgtaacaaagcctatcagaagctcaacacccttgctcttaaaaatgggataacgaaaaagtttatttgtgctggattggaagaaggtgggaaagatgcttgtcaaggcgattctggtggaccgttgatgctagtgaacaatagtagttggatagtgacgggagtggtgtcgttcggacacaagtgtgccgaagagggatttcctggtgtgtacacgcgtgtagtgagttacctagagtggatcgcgaaggttacgaactcgttagaccagacagtcactaactga

SEQ ID NO: 9 - DNA, 1203 bp, Artificial Sequence
  Limulus polyphemus factor B variant
atggcgtggatttgtgtgataacgttgtttgctttggcttctagtacgttgagtaataaagttagtagagtggggatcatctttcctaagacacagaacgataataaacagtgtacagcaaaaggtggattaaaagggtcctgcaagtccctcacagactgtcctgctgtcttggctacgttgaaggatagtttccctgtcgtttgctcttggaatggtcggtttcagcctattgtatgttgtcctgatgcagcagcaccaagtgtaaccacaacagttacaactattgtccctacaaaagaaacaaagattccaagattacatataccaggttgtggaaaaagaaaagtaaatgtagatattacaactattggacgttcggggtcaccaatacttcctcccatatctacttctcaagatttgaagggtgggagaggaatcattgctggaggtgtagaagctaaaattggcgcctggccttggatggcagctgtttttgtgaaaaattttggcattggcagattccattgtgctggtagcataatcagtagcaagtacattttgtctgctgcccactgcttcctcattggaggtcgaaagctgaccccaactcgcttagctgtccgcgtaggaggccactacgtaaagatgggtcaagaatatcatgtggaagatgtgattatccatcctgactacgtagaaagggagaattacaatgatattgctatcattgtgttaaaagaggaactgaattttactgatttggtccgtccaatctgtctccctgacccagaggcagtaacagattcattaaaaggcagaagggtgacagtagctggatggggtgatctggatttcgccggtccacgaagtcaagttctgcgcgaggttagtatccccgttgttccaatcggtgactgtaacaaagcctatcagaagctcaacacccttgctcttaaaaatgggataacgaaaaagtttatttgtgctggattggaagaaggtgggaaagatgcttgtcaaggcgattctggtggaccgttgatgctagtgaacaatagtagttggatagtgacgggagtggtgtcgttcggacacaagtgtgccgaagagggatttcctggtgtgtacacgcgtgtagtgagttacctagagtggatcgcgaaggttacgaactcgttagaccagacagtcactaactga

SEQ ID NO: 10 - protein, 400 aa, Artificial Sequence
  Limulus polyphemus factor B variant
MAWICVITLFALASSTLSNKVSRVGIIFPKTQNDNKQCTAKGGLKGSCKSLTDCPAVLATLKDSFPVVCSWNGRFQPIVCCPDAAAPSVTTTVTTIVPTKETKIPRLHIPGCGKRKVNVDITTIGRSGSPILPPISTSQDLKGGRGIIAGGVEAKIGAWPWMAAVFVKNFGIGRFHCAGSIISSKYILSAAHCFLIGGRKLTPTRLAVRVGGHYVKMGQEYHVEDVIIHPDYVERENYNDIAIIVLKEELNFTDLVRPICLPDPEAVTDSLKGRRVTVAGWGDLDFAGPRSQVLREVSIPVVPIGDCNKAYQKLNTLALKNGITKKFICAGLEEGGKDACQGDSGGPLMLVNNSSWIVTGVVSFGHKCAEEGFPGVYTRVVSYLEWIAKVTNSLDQTVTN

SEQ ID NO: 11 - DNA, 3060 bp, Tachypleus tridentatus
  Tachypleus tridentatus factor C
atggtcttagcgtcgtttttggtgtctggtttagttctagggatactagcccaacaaatgcgtccagttcagtccagaggagtagatctgggcttgtgtgatgaaacgaggttcgagtgtaagtgtggagatccaggctatgtgttcaacgtccctatgaaacaatgcacgtacttctatcgatggaggccttattgtaaaccatgtgatgacctggaggctaaggacatttgtccaaagtacaaacgatgtcaagagtgtaaggctggtcttgatagttgtgttacttgtccacctaacaaatatggtacttggtgtagcggtgaatgtcaatgtaagaatggaggtatctgtgaccagaggacaggagcttgtacctgtcgtgacagatatgaaggagcgcactgtgaaattctcaaaggttgtcctcttcttccatcggattctcaagttcaggaagtcagaaacccaccagataatccccaaactattgactacagctgttcaccagggttcaagcttaaaggcgtggcacgaattagctgtctcccaaatggacagtggagtagctttccacccaaatgtattcgagaatgtgccaaggtttcatctccagaacacgggaaagtgaatgctcctagtggcaatatgatagaaggggctactttacggttctcatgtgatagtccctactacttgattggtcaagaaacattaacctgccagggtaatggtcagtggagtggacaaataccacaatgtaagaagttggtcttctgtcctgaccttgatcctgtaaaccatgctgaacaccaggttaaaattggtgtggaacaaaaatatggtcagtttcctcaaggcactgaagtgacctatacgtgttcgggtaactacttcttgatgggttttaacaccttaaaatgtaaccctgatgggtcctggtcaggatcacagccatcctgtgttaaagtggcagacagagaggtcgactgtgacagtaaagctgtagacttcttggatgatgttggtgaacctgtcaggatccactgtcctgctggctgttctttgacagctggtactgtgtggggtacagccatataccacgaactttcctcagtgtgtcgtgcagccatccatgctggcaagcttccaaactctggaggggcggtgcatgtagtgaacaatggcccctactcggactttctgggtagtgacctgaatgggataaaatcggaagagttgaagtctcttgcccgcagttttcgatttgattatgtcagttcatccacagcaggtagatcaggatgtcctgatggatggtttgaggtagaagagaactgtgtgtacgttacatcaaaacagagagcctgggaaagagctcaaggtgtgtgtaccaatatggctgctcgtcttgctgtgctagacaaagatctaattccgagttccttgactgagactctacgagggaaagggttaacaaccacatggataggattgcacagactagatgctgagaagccctttgtttgggagctaatggatcgtagtaatgtggttctgaatgataacctaacattctgggcctctggcgaacctggaaatgaaactaactgtgtatatctggacatccgagatcagctgcagcctgtgtggaaaaccaagtcatgttttcagccctcaagctttgcttgcatgatggatttgtcagacagaaataaagccaaatgcgatgaccctggaccactggaaaatggacacgccacacttcatggacaaagtattgatgggttctatgctggttcttctataaggtacagctgtgaggttctccactacctcagtggaactgagaccgtaacttgtacaacaaatggcacatggagtgctcctaaacctcgatgtatcaaagtcatcacctgccaaaaccctcctgtaccatcatatggttctgtggaaatcaaacccccaagtcggacaaactcgatcagtcgtgttgggtcacctttcttgaggttgccacggttacccctcccattagccagagcagccaaacctcctccaaaacctagatcctcacaaccctctactgtggacttggcttctaaagttaaactacctgaaggtcattaccgggtagggtctcgagccatttacacgtgcgagtcgagatactacgaactacttggatctcaaggcagaagatgtgactctaatggaaactggagtggtcggcccgctagctgtattccagtttgtggacggtcagactctcctcgttctcctttcatctggaatgggaattctacagaaataggtcagtggccgtggcaggcaggaatctctcgatggcttgcagaccacaatatgtggtttctccagtgtggaggatccctattgaatgagaaatggatcgtcactgctgcccactgtgtcacctactctgctactgctgagataattgatcccagtcagtttaaaatctatctgggcaagtactaccgtgatgacagtagagacgatgactacgtacaagtaagagaggctctcgagatccacgtaaatcctaactacgaccccggcaatctcaactttgacatagccctaattcaactgaaaactcctgttactttgacaacacgagtccaaccaatctgtctgcctactgacatcacaacaagagaacacttgaaggagggaacattagcagtggtgacaggttggggtttgaatgaaaacaacacatattcagagatgattcaacaagctgtgctacctgttgttgcagcaagcacctgtgaagaggggtacaaggaagcagacttaccactgacagtaacagagaacatgttctgtgcaggttacaagaagggacgttatgatgcctgcagtggggacagtggaggaccattagtgtttgctgatgattcccgtaccgaaaggcggtgggtcttggaagggattgtcagctggggcagtcccagtggatgtggcaaggctaaccagtatgggggcttcactaaagttaacgtttttctatcatggattaggcagttcatttga

SEQ ID NO: 12 - protein, 1019 aa, Tachypleus tridentatus
  Tachypleus tridentatus factor C
MVLASFLVSGLVLGILAQQMRPVQSRGVDLGLCDETRFECKCGDPGYVFNVPMKQCTYFYRWRPYCKPCDDLEAKDICPKYKRCQECKAGLDSCVTCPPNKYGTWCSGECQCKNGGICDQRTGACTCRDRYEGAHCEILKGCPLLPSDSQVQEVRNPPDNPQTIDYSCSPGFKLKGVARISCLPNGQWSSFPPKCIRECAKVSSPEHGKVNAPSGNMIEGATLRFSCDSPYYLIGQETLTCQGNGQWSGQIPQCKKLVFCPDLDPVNHAEHQVKIGVEQKYGQFPQGTEVTYTCSGNYFLMGFNTLKCNPDGSWSGSQPSCVKVADREVDCDSKAVDFLDDVGEPVRIHCPAGCSLTAGTVWGTAIYHELSSVCRAAIHAGKLPNSGGAVHVVNNGPYSDFLGSDLNGIKSEELKSLARSFRFDYVSSSTAGRSGCPDGWFEVEENCVYVTSKQRAWERAQGVCTNMAARLAVLDKDLIPSSLTETLRGKGLTTTWIGLHRLDAEKPFVWELMDRSNVVLNDNLTFWASGEPGNETNCVYLDIRDQLQPVWKTKSCFQPSSFACMMDLSDRNKAKCDDPGPLENGHATLHGQSIDGFYAGSSIRYSCEVLHYLSGTETVTCTTNGTWSAPKPRCIKVITCQNPPVPSYGSVEIKPPSRTNSISRVGSPFLRLPRLPLPLARAAKPPPKPRSSQPSTVDLASKVKLPEGHYRVGSRAIYTCESRYYELLGSQGRRCDSNGNWSGRPASCIPVCGRSDSPRSPFIWNGNSTEIGQWPWQAGISRWLADHNMWFLQCGGSLLNEKWIVTAAHCVTYSATAEIIDPSQFKIYLGKYYRDDSRDDDYVQVREALEIHVNPNYDPGNLNFDIALIQLKTPVTLTTRVQPICLPTDITTREHLKEGTLAVVTGWGLNENNTYSEMIQQAVLPVVAASTCEEGYKEADLPLTVTENMFCAGYKKGRYDACSGDSGGPLVFADDSRTERRWVLEGIVSWGSPSGCGKANQYGGFTKVNVFLSWIRQFI

SEQ ID NO: 13 - DNA, 3063 bp, Limulus polyphemus
  Limulus polyphemus factor C
atggtactagcgtcgttcttggtgtctggtttagttctagggctattagcccaacaaatgcacccagttcagtccagaggagtagatctgggcttgtgtgatgacacgaggtttgagtgtaagtgtggagatccaggatacgtgttcaacgtccccgcgaagcaatgtacgtacttctatcgatggaggccttattgtaaaccatgtgacaaactggaggctaaagatgtgtgtcccaagtacaaacgatgtcaagagtgtagggctggtctcgacagttgtgtgagttgtccacctaacaaatatggaacttggtgtagcggtgagtgtcagtgtaagaatgggggtatttgtgatcagaggacaggagcttgtacatgtcgtgacagatatgaaggtgtgcattgtgaaatccttcaaggttgtcctcttcttcaatcggatccccaggttcaggaagtaaaaaatccaccaaatgatccacaaactattgactacagctgttcaccaggcttcaagcttaaaggcgtggcacgtatcacctgtcttccaaatgggcagtggagtagctttccacccaaatgtattcgagaatgttccatggtttcatctctagaacatggcaaagtaaactctcctagtgccgatctgatagaaggagctactttaaggttctcatgtgatagtccctactacttgattggtcaagaaacattaacctgccagggcaacggtcagtggagtgggcagataccacagtgtcagaaattggtcttctgccctgaccttgaccctgtaagccatgctgaacaccaggttaaaattggcctagaacaaaaatatggtcaatttcctcaaggcactgaagtaacctatacgtgtactggtaattacttcttgatgggtttggacaccttaaaatgtaaccctgatgggtcctggtcgggaacacagccgtcctgtgttaaagtggcagacagagaggtcaactgtgacagtaaagctgtggacttcttggatgatgttggcgaacctgtcaggatccactgtcctgctggctgttccttaactgctggtactgtatggggtacagccatatatcacgaactttcctcagtatgtcgtgcagctattcatgctggcaaggttccaaactctggaggtgcagtgcatgtagtgaacaacggtccgtactcagactttctggctagtgatctgaatgggataaaatcagacgagttgaagtctcttgctcagagtttccgattcgattatgtcagttcatcaacagcagggagaaagtcaggatgtcctgatggatggttcgagattgaggagaactgtgtgtacgttacatcgaaacagagagcctgggaaagagctcaaggtgtatgtaccaatatggccgctcgtcttgctgtgttagacaaagatgtaattccaagttccttgactgagactctacgagggaaagggttagcaacgacgtggattggactacacagattagatgctgataatcactttatttgggagctaatggatcgcagtagtgttgctttgaatgacagcctaacattctgggctcctggagaacctgggaatgaaactaactgtgtatatctggatatccaagatcagctacagccagtgtggaaaaccaagtcttgttttcaaccctcaagttttgtttgtatgatggatttgtcagacaagaacaaagccaaatgcaaagaccctggacctttggaaaacggacacgccaagcttcatggtcaaagtattgatggattttatgctgggtcttctgtaagatacagctgcgaggtcctccactacctcagtggaactgagacagtatcttgtacatcaaatggcacgtggagtgcccctaaacctcgatgtattaaagtcatcacctgccaaacccctcctgtaccatcctatggttctgtggacatcaaacccccaagtagaacaaactcaatcagtcgtgttgggtcgccattcttgaggttgccacggttacccctccctttagccagagcagccggacctcctccaaaacctagatccgcaccaccctctactgtggacctgtcttccaaggtcaaactgcctgaaggtcattaccgggtggggtctcaagccatttacacgtgcgagtcaagatactacgaactgcttggatctcaaggtagaagatgcgactctaatggaaagtggagtggtcgaccagcaagctgtataccagtttgtggacggtcagactctccccgttctcctttcatcgtcaatggaaattccaccgaaataggtcagtggccgtggcaggcaggaatctccagatggcttgcagatcataatatgtggtttcttcagtgtggaggagctctactgaatgagaaatggatcattactgcagcccactgtgtcacctactctgctactgccgagatcattgacccaagtcagtttaaattctacctgggcaaatactatcgagatgacagtaaggatgatgactacgtacaagtaagagaggctatcgagatccatgtgaatcctaactacgatcctggaaatctcaactttgacatagccctgattcaactgaagacttctgttgctctgaccacacgagtgcaaccaatatgtctgcctactgatctcactacaagagaaaacctgaaagagggagcgttagcggtggtgacaggatggggtttgaatgaaaacaacacatattcagagatgattcagcaagccgttctgcctgttgttgcagcaagcacctgtgaacaaggatatcaggactcgggcttgccactgacagtgacagagaacatgttctgtgcaggttacaagcaggggcgctatgatgcctgcagtggagacagtggaggaccattagtgtttgctgatgattcccgcaccgataggcggtgggtcctggaagggatcgtcagctggggcagccccaatggatgtggcaagtctaaccagtatgggggcttcactaaagttaacgtttttctatcgtggattcggcagttcatttga

SEQ ID NO: 14 - protein, 1020 aa, Limulus polyphemus
  Limulus polyphemus factor C
MVLASFLVSGLVLGLLAQQMHPVQSRGVDLGLCDDTRFECKCGDPGYVFNVPAKQCTYFYRWRPYCKPCDKLEAKDVCPKYKRCQECRAGLDSCVSCPPNKYGTWCSGECQCKNGGICDQRTGACTCRDRYEGVHCEILQGCPLLQSDPQVQEVKNPPNDPQTIDYSCSPGFKLKGVARITCLPNGQWSSFPPKCIRECSMVSSLEHGKVNSPSADLIEGATLRFSCDSPYYLIGQETLTCQGNGQWSGQIPQCQKLVFCPDLDPVSHAEHQVKIGLEQKYGQFPQGTEVTYTCTGNYFLMGLDTLKCNPDGSWSGTQPSCVKVADREVNCDSKAVDFLDDVGEPVRIHCPAGCSLTAGTVWGTAIYHELSSVCRAAIHAGKVPNSGGAVHVVNNGPYSDFLASDLNGIKSDELKSLAQSFRFDYVSSSTAGRKSGCPDGWFEIEENCVYVTSKQRAWERAQGVCTNMAARLAVLDKDVIPSSLTETLRGKGLATTWIGLHRLDADNHFIWELMDRSSVALNDSLTFWAPGEPGNETNCVYLDIQDQLQPVWKTKSCFQPSSFVCMMDLSDKNKAKCKDPGPLENGHAKLHGQSIDGFYAGSSVRYSCEVLHYLSGTETVSCTSNGTWSAPKPRCIKVITCQTPPVPSYGSVDIKPPSRTNSISRVGSPFLRLPRLPLPLARAAGPPPKPRSAPPSTVDLSSKVKLPEGHYRVGSQAIYTCESRYYELLGSQGRRCDSNGKWSGRPASCIPVCGRSDSPRSPFIVNGNSTEIGQWPWQAGISRWLADHNMWFLQCGGALLNEKWIITAAHCVTYSATAEIIDPSQFKFYLGKYYRDDSKDDDYVQVREAIEIHVNPNYDPGNLNFDIALIQLKTSVALTTRVQPICLPTDLTTRENLKEGALAVVTGWGLNENNTYSEMIQQAVLPVVAASTCEQGYQDSGLPLTVTENMFCAGYKQGRYDACSGDSGGPLVFADDSRTDRRWVLEGIVSWGSPNGCGKSNQYGGFTKVNVFLSWIRQFI

SEQ ID NO: 15 - DNA, 3060 bp, Carcinoscorpius rotundicauda
  Carcinoscorpius rotundicauda factor C
atggtcttagcgtcgtttttggtgtctggtttagttctagggctactagcccaaaaaatgcgcccagttcagtccaaaggagtagatctaggcttgtgtgatgaaacgaggttcgagtgtaagtgtggcgatccaggctatgtgttcaacattccagtgaaacaatgtacatacttttatcgatggaggccgtattgtaaaccatgtgatgacctggaggctaaggatatttgtccaaagtacaaacgatgtcaagagtgtaaggctggtcttgatagttgtgttacttgtccacctaacaaatatggtacttggtgtagcggtgaatgtcagtgtaagaatggaggtatctgtgaccagaggacaggagcttgtgcatgtcgtgacagatatgaaggggtgcactgtgaaattctcaaaggttgtcctcttcttccatcggattctcaggttcaggaagtcagaaatccaccagataatccccaaactattgactacagctgttcaccagggttcaagcttaagggtatggcacgaattagctgtctcccaaatggacagtggagtaactttccacccaaatgtattcgagaatgtgccatggtttcatctccagaacatgggaaagtgaatgctcttagtggtgatatgatagaaggggctactttacggttctcatgtgatagtccctactacttgattggtcaagaaacattaacctgtcagggtaatggtcagtggaatggacagataccacaatgtaagaacttggtcttctgtcctgacctggatcctgtaaaccatgctgaacacaaggttaaaattggtgtggaacaaaaatatggtcagtttcctcaaggcactgaagtgacctatacgtgttcgggtaactacttcttgatgggttttgacaccttaaaatgtaaccctgatgggtcttggtcaggatcacagccatcctgtgttaaagtggcagacagagaggtcgactgtgacagtaaagctgtagacttcttggatgatgttggtgaacctgtcaggatccactgtcctgctggctgttctttgacagctggtactgtgtggggtacagccatataccatgaactttcctcagtgtgtcgtgcagccatccatgctggcaagcttccaaactctggaggagcggtgcatgttgtgaacaatggcccctactcggactttctgggtagtgacctgaatgggataaaatcggaagagttgaagtctcttgcccggagtttccgattcgattatgtccgttcctccacagcaggtaaatcaggatgtcctgatggatggtttgaggtagacgagaactgtgtgtacgttacatcaaaacagagagcctgggaaagagctcaaggtgtgtgtaccaatatggctgctcgtcttgctgtgctggacaaagatgtaattccaaattcgttgactgagactctacgagggaaagggttaacaaccacgtggataggattgcacagactagatgctgagaagccctttatttgggagttaatggatcgtagtaatgtggttctgaatgataacctaacattctgggcctctggcgaacctggaaatgaaactaactgtgtatatatggacatccaagatcagttgcagtctgtgtggaaaaccaagtcatgttttcagccctcaagttttgcttgcatgatggatctgtcagacagaaataaagccaaatgcgatgatcctggatcactggaaaatggacacgccacacttcatggacaaagtattgatgggttctatgctggttcttctataaggtacagctgtgaggttctccactacctcagtggaactgaaaccgtaacttgtacaacaaatggcacatggagtgctcctaaacctcgatgtatcaaagtcatcacctgccaaaacccccctgtaccatcatatggttctgtggaaatcaaacccccaagtcggacaaactcgataagtcgtgttgggtcacctttcttgaggttgccacggttacccctcccattagctagagcagccaaacctcctccaaaacctagatcctcacaaccctctactgtggacttggcttctaaagttaaactacctgaaggtcattaccgggtagggtctcgagccatctacacgtgcgagtcgagatactacgaactacttggatctcaaggcagaagatgtgactctaatggaaactggagtggtcggccagcgagctgtattccagtttgtggacggtcagactctcctcgttctccttttatctggaatgggaattctacagaaataggtcagtggccgtggcaggcaggaatctctagatggcttgcagaccacaatatgtggtttctccagtgtggaggatctctattgaatgagaaatggatcgtcactgctgcccactgtgtcacctactctgctactgctgagattattgaccccaatcagtttaaaatgtatctgggcaagtactaccgtgatgacagtagagacgatgactatgtacaagtaagagaggctcttgagatccacgtgaatcctaactacgaccccggcaatctcaactttgacatagccctaattcaactgaaaactcctgttactttgacaacacgagtccaaccaatctgtctgcctactgacatcacaacaagagaacacttgaaggagggaacattagcagtggtgacaggttggggtttgaatgaaaacaacacctattcagagacgattcaacaagctgtgctacctgttgttgcagccagcacctgtgaagaggggtacaaggaagcagacttaccactgacagtaacagagaacatgttctgtgcaggttacaagaagggacgttatgatgcctgcagtggggacagtggaggacctttagtgtttgctgatgattcccgtaccgaaaggcggtgggtcttggaagggattgtcagctggggcagtcccagtggatgtggcaaggcgaaccagtacgggggcttcactaaagttaacgttttcctgtcatggattaggcagttcatttga

SEQ ID NO: 16 - protein, 1019 aa, Carcinoscorpius rotundicauda
  Carcinoscorpius rotundicauda factor C
MVLASFLVSGLVLGLLAQKMRPVQSKGVDLGLCDETRFECKCGDPGYVFNIPVKQCTYFYRWRPYCKPCDDLEAKDICPKYKRCQECKAGLDSCVTCPPNKYGTWCSGECQCKNGGICDQRTGACACRDRYEGVHCEILKGCPLLPSDSQVQEVRNPPDNPQTIDYSCSPGFKLKGMARISCLPNGQWSNFPPKCIRECAMVSSPEHGKVNALSGDMIEGATLRFSCDSPYYLIGQETLTCQGNGQWNGQIPQCKNLVFCPDLDPVNHAEHKVKIGVEQKYGQFPQGTEVTYTCSGNYFLMGFDTLKCNPDGSWSGSQPSCVKVADREVDCDSKAVDFLDDVGEPVRIHCPAGCSLTAGTVWGTAIYHELSSVCRAAIHAGKLPNSGGAVHVVNNGPYSDFLGSDLNGIKSEELKSLARSFRFDYVRSSTAGKSGCPDGWFEVDENCVYVTSKQRAWERAQGVCTNMAARLAVLDKDVIPNSLTETLRGKGLTTTWIGLHRLDAEKPFIWELMDRSNVVLNDNLTFWASGEPGNETNCVYMDIQDQLQSVWKTKSCFQPSSFACMMDLSDRNKAKCDDPGSLENGHATLHGQSIDGFYAGSSIRYSCEVLHYLSGTETVTCTTNGTWSAPKPRCIKVITCQNPPVPSYGSVEIKPPSRTNSISRVGSPFLRLPRLPLPLARAAKPPPKPRSSQPSTVDLASKVKLPEGHYRVGSRAIYTCESRYYELLGSQGRRCDSNGNWSGRPASCIPVCGRSDSPRSPFIWNGNSTEIGQWPWQAGISRWLADHNMWFLQCGGSLLNEKWIVTAAHCVTYSATAEIIDPNQFKMYLGKYYRDDSRDDDYVQVREALEIHVNPNYDPGNLNFDIALIQLKTPVTLTTRVQPICLPTDITTREHLKEGTLAVVTGWGLNENNTYSETIQQAVLPVVAASTCEEGYKEADLPLTVTENMFCAGYKKGRYDACSGDSGGPLVFADDSRTERRWVLEGIVSWGSPSGCGKANQYGGFTKVNVFLSWIRQFI

SEQ ID NO: 17 - DNA, 1128 bp, Tachypleus tridentatus
  Tachypleus tridentatus pro-clotting enzyme
atgttggtgaataacgtgttttcactactgtgtttcccactcttgatgtctgtggttagatgcagtactctcagcagacagcgtagacagtttgttttccctgacgaggaagaactttgctcaaaccgatttactgaagaaggaacatgcaaaaatgtcttggattgtagaatacttttacaaaaaaatgattataatttactcaaagaatcaatatgcggctttgaaggcataacacccaaagtttgttgtccgaaatcaagccatgtaatttcaagtacacaggcacctccagaaaccactacgactgaacgcccaccaaaacagataccacccaatcttcctgaagtgtgtggaattcacaatactacaactaccaggattattggaggtcgggaagcacctattggagcctggccgtggatgactgctgtctacataaaacaaggaggaatcagaagtgttcagtgtggtggcgcacttgtcactaacaggcacgtgattacagcttcgcactgtgttgtaaacagtgcaggaacagatgtgatgccagctgatgtattctcggttcgtctgggtgaacacaatttatacagtaccgatgacgattcgaatccaatagattttgcagttacgtcggtgaaacatcacgaacactttgtactcgcgacgtatttgaatgacatcgcaattctaacgttaaatgacacagttacgtttacagacagaattcgacccatttgtctaccttatcgtaagttgagatacgatgatctagcaatgagaaaaccgtttatcactggatggggaacaacagcatttaacggcccatctagtgcagtgttgagagaagtacagttaccaatatgggaacacgaggcctgtagacaggcctacgagaaggatttaaatattacaaacgtgtatatgtgtgctggctttgcagatggcgggaaggatgcttgccagggtgattctggaggtccaatgatgttgcctgttaaaaccggagagttttatctcattggaattgtgtctttcggaaagaaatgcgcattgcctggatttcctggggtttacacaaaagtgacagagtttttagattggattgcagaacatatggtgtag

SEQ ID NO: 18 - protein, 375 aa, Tachypleus tridentatus
  Tachypleus tridentatus pro-clotting enzyme
MLVNNVFSLLCFPLLMSVVRCSTLSRQRRQFVFPDEEELCSNRFTEEGTCKNVLDCRILLQKNDYNLLKESICGFEGITPKVCCPKSSHVISSTQAPPETTTTERPPKQIPPNLPEVCGIHNTTTTRIIGGREAPIGAWPWMTAVYIKQGGIRSVQCGGALVTNRHVITASHCVVNSAGTDVMPADVFSVRLGEHNLYSTDDDSNPIDFAVTSVKHHEHFVLATYLNDIAILTLNDTVTFTDRIRPICLPYRKLRYDDLAMRKPFITGWGTTAFNGPSSAVLREVQLPIWEHEACRQAYEKDLNITNVYMCAGFADGGKDACQGDSGGPMMLPVKTGEFYLIGIVSFGKKCALPGFPGVYTKVTEFLDWIAEHMV

SEQ ID NO: 19 - DNA, 1128 bp, Limulus polyphemus
  Limulus polyphemus pro-clotting enzyme
atgttggtgaataacatgttttcattgctgtgtttcccactcctgatgtctatgtttagctgcagtagtctcggcagacagcgtagacagtttgttttccccgatgatgaagaatcatgctcaaaccgatttactaacgatggaatatgtaaagatgttttgaattgtagagatcttttacaaaaaaatgattataatttactgaaagaatcaatatgcggttttgaaggcataacacccaaagtttgttgtccgaaacaaagtattgtaaatccaataacagaagcacctccaaaaaccactacaactgaacgaccgccaatacggataccatccaatcttcctaaacagtgtggaaatcgtaatattacaactaccaggattattggagggcaggaagcaacacctggagcctggccctggatggctgctgtctatatcaaacaaggaggaatcagaagtgttcagtgtggaggtgcgcttgtcaccaacaggcacgtgattacagcatcgcactgtgttgtaaacagtttaggaacagatgtgatgcgagctgacgtattctcggttcgcctaggtgaacacaatttatatagcaccaatgacagttcagatccaattgattttgcagttacgtcagtgaaacatcatgaaaactttgtgctcgcgacgtatttgaatgatatcgcaattctgaagttaaacgacactgttacgtttacgcacaaaattaaaccaatttgtctaccttatgaaagcttaaggtatgaggatctagcaatgagaaacccatttgtcgccggatggggaacaacagcatttaatggcccatctagtgcagtattacgagaagtgcagttaccaatatggggacacgagccctgcaggcaggcctacgagaaggatttaaatattacaaacgtgtatatgtgtgctgggtatgcagatggcggtaaagatgcttgccagggtgattctggaggtccaatgatgttgcctgataaaagcgggaacttttatctcgttggaattgtgtctttcggaaagaaatgcgcgttgcctggatttcctggggtttacacaaaagtgaccgaatttttagattggattgcagtaaatatggtgtag

SEQ ID NO: 20 - protein, 375 aa, Limulus polyphemus
  Limulus polyphemus pro-clotting enzyme
MLVNNMFSLLCFPLLMSMFSCSSLGRQRRQFVFPDDEESCSNRFTNDGICKDVLNCRDLLQKNDYNLLKESICGFEGITPKVCCPKQSIVNPITEAPPKTTTTERPPIRIPSNLPKQCGNRNITTTRIIGGQEATPGAWPWMAAVYIKQGGIRSVQCGGALVTNRHVITASHCVVNSLGTDVMRADVFSVRLGEHNLYSTNDSSDPIDFAVTSVKHHENFVLATYLNDIAILKLNDTVTFTHKIKPICLPYESLRYEDLAMRNPFVAGWGTTAFNGPSSAVLREVQLPIWGHEPCRQAYEKDLNITNVYMCAGYADGGKDACQGDSGGPMMLPDKSGNFYLVGIVSFGKKCALPGFPGVYTKVTEFLDWIAVNMV

SEQ ID NO: 21 - DNA, 27 bp, Artificial Sequence
  designed primer (primer 1)
gggaccggtagaggagtagatctgggc

SEQ ID NO: 22 - DNA, 30 bp, Artificial Sequence
  designed primer (primer 2)
gggctcgagtcattaaatgaactgcctaat

SEQ ID NO: 23 - DNA, 39 bp, Artificial Sequence
  designed primer (primer 3)
ggggaattcaagcttgccaccatggtcttagcgtcgttt

SEQ ID NO: 24 - DNA, 49 bp, Artificial Sequence
  designed primer (primer 4)
gccctcgatgtgatggtgatggtggtgggactgaactggacgcatttgt

SEQ ID NO: 25 - DNA, 28 bp, Artificial Sequence
  designed primer (primer 5)
agaagaggagtagatctgggcttgtgtg

SEQ ID NO: 26 - DNA, 30 bp, Artificial Sequence
  designed primer (primer 6)
gggaccggtcaccaccatcaccatcacatc

SEQ ID NO: 27 - DNA, 30 bp, Artificial Sequence
  designed primer (primer 7)
tctagattatcaaatgaactgcctaatcca

SEQ ID NO: 28 - DNA, 18 bp, Artificial Sequence
  BGH reverse primer
tagaaggcacagtcgagg

SEQ ID NO: 29 - DNA, 24 bp, Artificial Sequence
  designed primer (primer 8)
agcctctgctaaccatgttcatgc

SEQ ID NO: 30 - DNA, 27 bp, Artificial Sequence
  designed primer (primer 9)
gggaccggtgtgggggtcctcttcccc

SEQ ID NO: 31 - DNA, 30 bp, Artificial Sequence
  designed primer (primer 10)
gggctcgagttagttagtgacggcatgatc

SEQ ID NO: 32 - DNA, 35 bp, Artificial Sequence
  designed primer (primer 11)
cttccttatcggaggtcgaaagttgaccccaactc

SEQ ID NO: 33 - DNA, 35 bp, Artificial Sequence
  designed primer (primer 12)
cagtgggcagctgacaaaatgtacttgttactgat

SEQ ID NO: 34 - DNA, 57 bp, Artificial Sequence
  designed primer (primer 13)
gggaccggtcaccaccatcaccatcacatcgagggcagaagaggagtagatctgggc

SEQ ID NO: 35 - DNA, 35 bp, Artificial Sequence
  designed primer (primer 14)
gggctcgagtcaaatgaactgccgaatccacgata

SEQ ID NO: 36 - DNA, 39 bp, Artificial Sequence
  designed primer (primer 15)
ggggaattcaagcttgccaccatggcgtggatttgtgtg

SEQ ID NO: 37 - DNA, 33 bp, Artificial Sequence
  designed primer (primer 16)
acctccaatgaggaagcagtgggcagcagacaa

SEQ ID NO: 38 - DNA, 33 bp, Artificial Sequence
  designed primer (primer 17)
ttgtctgctgcccactgcttcctcattggaggt

SEQ ID NO: 39 - DNA, 35 bp, Artificial Sequence
  designed primer (primer 18)
gggctcgagtcagttagtgactgcctggtctaacg

SEQ ID NO: 40 - DNA, 48 bp, Artificial Sequence
  designed primer (primer 19)
gggctcgagtcagtgatggtgatggtggtggttagtgactgcctggtc

SEQ ID NO: 41 - DNA, 35 bp, Artificial Sequence
  designed primer (primer 20)
gggaccggtgtggggatcatctttcctaagacaca

SEQ ID NO: 42 - DNA, 23 bp, Artificial Sequence
  designed primer (primer 21)
caccagccaccaccttctgatag